European Patent Application EP 4 793 354 A2, published August 19, 2026. Title: MISMATCHED siRNA, siRNA CONJUGATE, PHARMACEUTICAL COMPOSITION AND USE THEREOF. Applicant: CHENGDU GOWELL BIOPHARMACEUTICAL CO., LTD. The sequence listing filed with the application follows.

SEQUENCE LISTING (52 sequences)

SEQ ID NO: 1 - RNA, 21 nt, synthetic construct
  source 1..21: mol_type = other RNA
  modified_base 1..6: mod_base = OTHER; note = 2'-O-methyl nucleotide
  modified_base 1^2: mod_base = OTHER; note = Phosphorothioate Linkage
  modified_base 2^3: mod_base = OTHER; note = Phosphorothioate Linkage
  modified_base 7: mod_base = OTHER; note = 2'-Fluoro nucleotide
  modified_base 8: mod_base = OTHER; note = 2'-O-methyl nucleotide
  modified_base 9: mod_base = OTHER; note = 2'-Fluoro nucleotide
  modified_base 10: mod_base = OTHER; note = 2'-Fluoro nucleotide
  modified_base 11: mod_base = OTHER; note = 2'-Fluoro nucleotide
  modified_base 12: mod_base = OTHER; note = 2'-O-methyl nucleotide
  modified_base 13: mod_base = OTHER; note = 2'-Fluoro nucleotide
  modified_base 14..21: mod_base = OTHER; note = 2'-O-methyl nucleotide
  modified_base 19^20: mod_base = OTHER; note = Phosphorothioate Linkage
  modified_base 20^21: mod_base = OTHER; note = Phosphorothioate Linkage
  modified_base 21: mod_base = OTHER; note = GalNAc(L96) modification
  misc_feature 1..21: note = siRNA
agccaaaatcaagatttgcta

SEQ ID NO: 2 - RNA, 23 nt, synthetic construct
  source 1..23: mol_type = other RNA
  modified_base 1: mod_base = OTHER; note = 2'-O-methyl nucleotide
  modified_base 1^2: mod_base = OTHER; note = Phosphorothioate Linkage
  modified_base 2: mod_base = OTHER; note = 2'-Fluoro nucleotide
  modified_base 2^3: mod_base = OTHER; note = Phosphorothioate Linkage
  modified_base 3: mod_base = OTHER; note = 2'-O-methyl nucleotide
  modified_base 4: mod_base = OTHER; note = 2'-Fluoro nucleotide
  modified_base 5: mod_base = OTHER; note = 2'-O-methyl nucleotide
  modified_base 6: mod_base = OTHER; note = 2'-Fluoro nucleotide
  modified_base 7..13: mod_base = OTHER; note = 2'-O-methyl nucleotide
  modified_base 14: mod_base = OTHER; note = 2'-Fluoro nucleotide
  modified_base 15: mod_base = OTHER; note = 2'-O-methyl nucleotide
  modified_base 16: mod_base = OTHER; note = 2'-Fluoro nucleotide
  modified_base 17..23: mod_base = OTHER; note = 2'-O-methyl nucleotide
  modified_base 21^22: mod_base = OTHER; note = Phosphorothioate Linkage
  modified_base 22^23: mod_base = OTHER; note = Phosphorothioate Linkage
  misc_feature 1..23: note = siRNA
tagcaaatcttgattttggctct

SEQ ID NO: 3 - RNA, 21 nt, synthetic construct
  source 1..21: mol_type = other RNA
  modified_base 1..6: mod_base = OTHER; note = 2'-O-methyl nucleotide
  modified_base 1^2: mod_base = OTHER; note = Phosphorothioate Linkage
  modified_base 2^3: mod_base = OTHER; note = Phosphorothioate Linkage
  modified_base 7: mod_base = OTHER; note = 2'-Fluoro nucleotide
  modified_base 8: mod_base = OTHER; note = 2'-O-methyl nucleotide
  modified_base 9: mod_base = OTHER; note = 2'-Fluoro nucleotide
  modified_base 10: mod_base = OTHER; note = 2'-Fluoro nucleotide
  modified_base 11: mod_base = OTHER; note = 2'-Fluoro nucleotide
  modified_base 12: mod_base = OTHER; note = 2'-O-methyl nucleotide
  modified_base 13: mod_base = OTHER; note = 2'-Fluoro nucleotide
  modified_base 14..21: mod_base = OTHER; note = 2'-O-methyl nucleotide
  modified_base 19^20: mod_base = OTHER; note = Phosphorothioate Linkage
  modified_base 20^21: mod_base = OTHER; note = Phosphorothioate Linkage
  modified_base 21: mod_base = OTHER; note = GalNAc(L96) modification
  misc_feature 1..21: note = siRNA
tgccaaaatcaagatttgcta

SEQ ID NO: 4 - RNA, 23 nt, synthetic construct
  source 1..23: mol_type = other RNA
  modified_base 1: mod_base = OTHER; note = 2'-O-methyl nucleotide
  modified_base 1^2: mod_base = OTHER; note = Phosphorothioate Linkage
  modified_base 2: mod_base = OTHER; note = 2'-Fluoro nucleotide
  modified_base 2^3: mod_base = OTHER; note = Phosphorothioate Linkage
  modified_base 3: mod_base = OTHER; note = 2'-O-methyl nucleotide
  modified_base 4: mod_base = OTHER; note = 2'-Fluoro nucleotide
  modified_base 5: mod_base = OTHER; note = 2'-O-methyl nucleotide
  modified_base 6: mod_base = OTHER; note = 2'-Fluoro nucleotide
  modified_base 7..13: mod_base = OTHER; note = 2'-O-methyl nucleotide
  modified_base 14: mod_base = OTHER; note = 2'-Fluoro nucleotide
  modified_base 15: mod_base = OTHER; note = 2'-O-methyl nucleotide
  modified_base 16: mod_base = OTHER; note = 2'-Fluoro nucleotide
  modified_base 17..23: mod_base = OTHER; note = 2'-O-methyl nucleotide
  modified_base 21^22: mod_base = OTHER; note = Phosphorothioate Linkage
  modified_base 22^23: mod_base = OTHER; note = Phosphorothioate Linkage
  misc_feature 1..23: note = siRNA
tagcaaatcttgattttggcact

SEQ ID NO: 5 - RNA, 21 nt, synthetic construct
  source 1..21: mol_type = other RNA
  modified_base 1..6: mod_base = OTHER; note = 2'-O-methyl nucleotide
  modified_base 1^2: mod_base = OTHER; note = Phosphorothioate Linkage
  modified_base 2^3: mod_base = OTHER; note = Phosphorothioate Linkage
  modified_base 7: mod_base = OTHER; note = 2'-Fluoro nucleotide
  modified_base 8: mod_base = OTHER; note = 2'-O-methyl nucleotide
  modified_base 9: mod_base = OTHER; note = 2'-Fluoro nucleotide
  modified_base 10: mod_base = OTHER; note = 2'-Fluoro nucleotide
  modified_base 11: mod_base = OTHER; note = 2'-Fluoro nucleotide
  modified_base 12: mod_base = OTHER; note = 2'-O-methyl nucleotide
  modified_base 13: mod_base = OTHER; note = 2'-Fluoro nucleotide
  modified_base 14..21: mod_base = OTHER; note = 2'-O-methyl nucleotide
  modified_base 19^20: mod_base = OTHER; note = Phosphorothioate Linkage
  modified_base 20^21: mod_base = OTHER; note = Phosphorothioate Linkage
  modified_base 21: mod_base = OTHER; note = GalNAc(L96) modification
  misc_feature 1..21: note = siRNA
tcccaaaatcaagatttgcta

SEQ ID NO: 6 - RNA, 23 nt, synthetic construct
  source 1..23: mol_type = other RNA
  modified_base 1: mod_base = OTHER; note = 2'-O-methyl nucleotide
  modified_base 1^2: mod_base = OTHER; note = Phosphorothioate Linkage
  modified_base 2: mod_base = OTHER; note = 2'-Fluoro nucleotide
  modified_base 2^3: mod_base = OTHER; note = Phosphorothioate Linkage
  modified_base 3: mod_base = OTHER; note = 2'-O-methyl nucleotide
  modified_base 4: mod_base = OTHER; note = 2'-Fluoro nucleotide
  modified_base 5: mod_base = OTHER; note = 2'-O-methyl nucleotide
  modified_base 6: mod_base = OTHER; note = 2'-Fluoro nucleotide
  modified_base 7..13: mod_base = OTHER; note = 2'-O-methyl nucleotide
  modified_base 14: mod_base = OTHER; note = 2'-Fluoro nucleotide
  modified_base 15: mod_base = OTHER; note = 2'-O-methyl nucleotide
  modified_base 16: mod_base = OTHER; note = 2'-Fluoro nucleotide
  modified_base 17..23: mod_base = OTHER; note = 2'-O-methyl nucleotide
  modified_base 21^22: mod_base = OTHER; note = Phosphorothioate Linkage
  modified_base 22^23: mod_base = OTHER; note = Phosphorothioate Linkage
  misc_feature 1..23: note = siRNA
tagcaaatcttgattttgggact

SEQ ID NO: 7 - RNA, 21 nt, synthetic construct
  source 1..21: mol_type = other RNA
  modified_base 1..6: mod_base = OTHER; note = 2'-O-methyl nucleotide
  modified_base 1^2: mod_base = OTHER; note = Phosphorothioate Linkage
  modified_base 2^3: mod_base = OTHER; note = Phosphorothioate Linkage
  modified_base 7: mod_base = OTHER; note = 2'-Fluoro nucleotide
  modified_base 8: mod_base = OTHER; note = 2'-O-methyl nucleotide
  modified_base 9: mod_base = OTHER; note = 2'-Fluoro nucleotide
  modified_base 10: mod_base = OTHER; note = 2'-Fluoro nucleotide
  modified_base 11: mod_base = OTHER; note = 2'-Fluoro nucleotide
  modified_base 12: mod_base = OTHER; note = 2'-O-methyl nucleotide
  modified_base 13: mod_base = OTHER; note = 2'-Fluoro nucleotide
  modified_base 14..21: mod_base = OTHER; note = 2'-O-methyl nucleotide
  modified_base 19^20: mod_base = OTHER; note = Phosphorothioate Linkage
  modified_base 20^21: mod_base = OTHER; note = Phosphorothioate Linkage
  modified_base 21: mod_base = OTHER; note = GalNAc(L96) modification
  misc_feature 1..21: note = siRNA
tcgcaaaatcaagatttgcta

SEQ ID NO: 8 - RNA, 23 nt, synthetic construct
  source 1..23: mol_type = other RNA
  modified_base 1: mod_base = OTHER; note = 2'-O-methyl nucleotide
  modified_base 1^2: mod_base = OTHER; note = Phosphorothioate Linkage
  modified_base 2: mod_base = OTHER; note = 2'-Fluoro nucleotide
  modified_base 2^3: mod_base = OTHER; note = Phosphorothioate Linkage
  modified_base 3: mod_base = OTHER; note = 2'-O-methyl nucleotide
  modified_base 4: mod_base = OTHER; note = 2'-Fluoro nucleotide
  modified_base 5: mod_base = OTHER; note = 2'-O-methyl nucleotide
  modified_base 6: mod_base = OTHER; note = 2'-Fluoro nucleotide
  modified_base 7..13: mod_base = OTHER; note = 2'-O-methyl nucleotide
  modified_base 14: mod_base = OTHER; note = 2'-Fluoro nucleotide
  modified_base 15: mod_base = OTHER; note = 2'-O-methyl nucleotide
  modified_base 16: mod_base = OTHER; note = 2'-Fluoro nucleotide
  modified_base 17..23: mod_base = OTHER; note = 2'-O-methyl nucleotide
  modified_base 21^22: mod_base = OTHER; note = Phosphorothioate Linkage
  modified_base 22^23: mod_base = OTHER; note = Phosphorothioate Linkage
  misc_feature 1..23: note = siRNA
tagcaaatcttgattttgcgact

SEQ ID NO: 9 - RNA, 21 nt, synthetic construct
  source 1..21: mol_type = other RNA
  modified_base 1..2: mod_base = OTHER; note = 2'-O-methyl nucleotide
  modified_base 1^2: mod_base = OTHER; note = Phosphorothioate Linkage
  modified_base 2^3: mod_base = OTHER; note = Phosphorothioate Linkage
  modified_base 3: mod_base = OTHER; note = 2'-Fluoro nucleotide
  modified_base 4..6: mod_base = OTHER; note = 2'-O-methyl nucleotide
  modified_base 7: mod_base = OTHER; note = 2'-Fluoro nucleotide
  modified_base 8: mod_base = OTHER; note = 2'-O-methyl nucleotide
  modified_base 9: mod_base = OTHER; note = 2'-Fluoro nucleotide
  modified_base 10: mod_base = OTHER; note = 2'-Fluoro nucleotide
  modified_base 11: mod_base = OTHER; note = 2'-Fluoro nucleotide
  modified_base 12..21: mod_base = OTHER; note = 2'-O-methyl nucleotide
  modified_base 21: mod_base = OTHER; note = GalNAc(L96) modification
  misc_feature 1..21: note = siRNA
agccaaaatcaagatttgcta

SEQ ID NO: 10 - RNA, 23 nt, synthetic construct
  source 1..23: mol_type = other RNA
  modified_base 1: mod_base = OTHER; note = 2'-O-methyl nucleotide
  modified_base 1^2: mod_base = OTHER; note = Phosphorothioate Linkage
  modified_base 2: mod_base = OTHER; note = 2'-Fluoro nucleotide
  modified_base 2^3: mod_base = OTHER; note = Phosphorothioate Linkage
  modified_base 3..5: mod_base = OTHER; note = 2'-O-methyl nucleotide
  modified_base 6: mod_base = OTHER; note = 2'-Fluoro nucleotide
  modified_base 7..9: mod_base = OTHER; note = 2'-O-methyl nucleotide
  modified_base 10: mod_base = OTHER; note = 2'-Fluoro nucleotide
  modified_base 11..13: mod_base = OTHER; note = 2'-O-methyl nucleotide
  modified_base 14: mod_base = OTHER; note = 2'-Fluoro nucleotide
  modified_base 15: mod_base = OTHER; note = 2'-O-methyl nucleotide
  modified_base 16: mod_base = OTHER; note = 2'-Fluoro nucleotide
  modified_base 17..23: mod_base = OTHER; note = 2'-O-methyl nucleotide
  modified_base 21^22: mod_base = OTHER; note = Phosphorothioate Linkage
  modified_base 22^23: mod_base = OTHER; note = Phosphorothioate Linkage
  misc_feature 1..23: note = siRNA
tagcaaatcttgattttggctct

SEQ ID NO: 11 - RNA, 21 nt, synthetic construct
  source 1..21: mol_type = other RNA
  modified_base 1..2: mod_base = OTHER; note = 2'-O-methyl nucleotide
  modified_base 1^2: mod_base = OTHER; note = Phosphorothioate Linkage
  modified_base 2^3: mod_base = OTHER; note = Phosphorothioate Linkage
  modified_base 3: mod_base = OTHER; note = 2'-Fluoro nucleotide
  modified_base 4..6: mod_base = OTHER; note = 2'-O-methyl nucleotide
  modified_base 7: mod_base = OTHER; note = 2'-Fluoro nucleotide
  modified_base 8: mod_base = OTHER; note = 2'-O-methyl nucleotide
  modified_base 9: mod_base = OTHER; note = 2'-Fluoro nucleotide
  modified_base 10: mod_base = OTHER; note = 2'-Fluoro nucleotide
  modified_base 11: mod_base = OTHER; note = 2'-Fluoro nucleotide
  modified_base 12..21: mod_base = OTHER; note = 2'-O-methyl nucleotide
  modified_base 21: mod_base = OTHER; note = GalNAc(L96) modification
  misc_feature 1..21: note = siRNA
tgccaaaatcaagatttgcta

SEQ ID NO: 12 - RNA, 23 nt, synthetic construct
  source 1..23: mol_type = other RNA
  modified_base 1: mod_base = OTHER; note = 2'-O-methyl nucleotide
  modified_base 1^2: mod_base = OTHER; note = Phosphorothioate Linkage
  modified_base 2: mod_base = OTHER; note = 2'-Fluoro nucleotide
  modified_base 2^3: mod_base = OTHER; note = Phosphorothioate Linkage
  modified_base 3..5: mod_base = OTHER; note = 2'-O-methyl nucleotide
  modified_base 6: mod_base = OTHER; note = 2'-Fluoro nucleotide
  modified_base 7..9: mod_base = OTHER; note = 2'-O-methyl nucleotide
  modified_base 10: mod_base = OTHER; note = 2'-Fluoro nucleotide
  modified_base 11..13: mod_base = OTHER; note = 2'-O-methyl nucleotide
  modified_base 14: mod_base = OTHER; note = 2'-Fluoro nucleotide
  modified_base 15: mod_base = OTHER; note = 2'-O-methyl nucleotide
  modified_base 16: mod_base = OTHER; note = 2'-Fluoro nucleotide
  modified_base 17..23: mod_base = OTHER; note = 2'-O-methyl nucleotide
  modified_base 21^22: mod_base = OTHER; note = Phosphorothioate Linkage
  modified_base 22^23: mod_base = OTHER; note = Phosphorothioate Linkage
  misc_feature 1..23: note = siRNA
tagcaaatcttgattttggcact

SEQ ID NO: 13 - RNA, 21 nt, synthetic construct
  source 1..21: mol_type = other RNA
  modified_base 1..2: mod_base = OTHER; note = 2'-O-methyl nucleotide
  modified_base 1^2: mod_base = OTHER; note = Phosphorothioate Linkage
  modified_base 2^3: mod_base = OTHER; note = Phosphorothioate Linkage
  modified_base 3: mod_base = OTHER; note = 2'-Fluoro nucleotide
  modified_base 4..6: mod_base = OTHER; note = 2'-O-methyl nucleotide
  modified_base 7: mod_base = OTHER; note = 2'-Fluoro nucleotide
  modified_base 8: mod_base = OTHER; note = 2'-O-methyl nucleotide
  modified_base 9: mod_base = OTHER; note = 2'-Fluoro nucleotide
  modified_base 10: mod_base = OTHER; note = 2'-Fluoro nucleotide
  modified_base 11: mod_base = OTHER; note = 2'-Fluoro nucleotide
  modified_base 12..21: mod_base = OTHER; note = 2'-O-methyl nucleotide
  modified_base 21: mod_base = OTHER; note = GalNAc(L96) modification
  misc_feature 1..21: note = siRNA
acccaaaatcaagatttgcta

SEQ ID NO: 14 - RNA, 23 nt, synthetic construct
  source 1..23: mol_type = other RNA
  modified_base 1: mod_base = OTHER; note = 2'-O-methyl nucleotide
  modified_base 1^2: mod_base = OTHER; note = Phosphorothioate Linkage
  modified_base 2: mod_base = OTHER; note = 2'-Fluoro nucleotide
  modified_base 2^3: mod_base = OTHER; note = Phosphorothioate Linkage
  modified_base 3..5: mod_base = OTHER; note = 2'-O-methyl nucleotide
  modified_base 6: mod_base = OTHER; note = 2'-Fluoro nucleotide
  modified_base 7..9: mod_base = OTHER; note = 2'-O-methyl nucleotide
  modified_base 10: mod_base = OTHER; note = 2'-Fluoro nucleotide
  modified_base 11..13: mod_base = OTHER; note = 2'-O-methyl nucleotide
  modified_base 14: mod_base = OTHER; note = 2'-Fluoro nucleotide
  modified_base 15: mod_base = OTHER; note = 2'-O-methyl nucleotide
  modified_base 16: mod_base = OTHER; note = 2'-Fluoro nucleotide
  modified_base 17..23: mod_base = OTHER; note = 2'-O-methyl nucleotide
  modified_base 21^22: mod_base = OTHER; note = Phosphorothioate Linkage
  modified_base 22^23: mod_base = OTHER; note = Phosphorothioate Linkage
  misc_feature 1..23: note = siRNA
tagcaaatcttgattttgggtct

SEQ ID NO: 15 - RNA, 21 nt, synthetic construct
  source 1..21: mol_type = other RNA
  modified_base 1..2: mod_base = OTHER; note = 2'-O-methyl nucleotide
  modified_base 1^2: mod_base = OTHER; note = Phosphorothioate Linkage
  modified_base 2^3: mod_base = OTHER; note = Phosphorothioate Linkage
  modified_base 3: mod_base = OTHER; note = 2'-Fluoro nucleotide
  modified_base 4..6: mod_base = OTHER; note = 2'-O-methyl nucleotide
  modified_base 7: mod_base = OTHER; note = 2'-Fluoro nucleotide
  modified_base 8: mod_base = OTHER; note = 2'-O-methyl nucleotide
  modified_base 9: mod_base = OTHER; note = 2'-Fluoro nucleotide
  modified_base 10: mod_base = OTHER; note = 2'-Fluoro nucleotide
  modified_base 11: mod_base = OTHER; note = 2'-Fluoro nucleotide
  modified_base 12..21: mod_base = OTHER; note = 2'-O-methyl nucleotide
  modified_base 21: mod_base = OTHER; note = GalNAc(L96) modification
  misc_feature 1..21: note = siRNA
aggcaaaatcaagatttgcta

SEQ ID NO: 16 - RNA, 23 nt, synthetic construct
  source 1..23: mol_type = other RNA
  modified_base 1: mod_base = OTHER; note = 2'-O-methyl nucleotide
  modified_base 1^2: mod_base = OTHER; note = Phosphorothioate Linkage
  modified_base 2: mod_base = OTHER; note = 2'-Fluoro nucleotide
  modified_base 2^3: mod_base = OTHER; note = Phosphorothioate Linkage
  modified_base 3..5: mod_base = OTHER; note = 2'-O-methyl nucleotide
  modified_base 6: mod_base = OTHER; note = 2'-Fluoro nucleotide
  modified_base 7..9: mod_base = OTHER; note = 2'-O-methyl nucleotide
  modified_base 10: mod_base = OTHER; note = 2'-Fluoro nucleotide
  modified_base 11..13: mod_base = OTHER; note = 2'-O-methyl nucleotide
  modified_base 14: mod_base = OTHER; note = 2'-Fluoro nucleotide
  modified_base 15: mod_base = OTHER; note = 2'-O-methyl nucleotide
  modified_base 16: mod_base = OTHER; note = 2'-Fluoro nucleotide
  modified_base 17..23: mod_base = OTHER; note = 2'-O-methyl nucleotide
  modified_base 21^22: mod_base = OTHER; note = Phosphorothioate Linkage
  modified_base 22^23: mod_base = OTHER; note = Phosphorothioate Linkage
  misc_feature 1..23: note = siRNA
tagcaaatcttgattttgcctct

SEQ ID NO: 17 - RNA, 21 nt, synthetic construct
  source 1..21: mol_type = other RNA
  modified_base 1..6: mod_base = OTHER; note = 2'-O-methyl nucleotide
  modified_base 1^2: mod_base = OTHER; note = Phosphorothioate Linkage
  modified_base 2^3: mod_base = OTHER; note = Phosphorothioate Linkage
  modified_base 7: mod_base = OTHER; note = 2'-Fluoro nucleotide
  modified_base 8: mod_base = OTHER; note = 2'-O-methyl nucleotide
  modified_base 9: mod_base = OTHER; note = 2'-Fluoro nucleotide
  modified_base 10: mod_base = OTHER; note = 2'-Fluoro nucleotide
  modified_base 11: mod_base = OTHER; note = 2'-Fluoro nucleotide
  modified_base 12: mod_base = OTHER; note = 2'-O-methyl nucleotide
  modified_base 13: mod_base = OTHER; note = 2'-Fluoro nucleotide
  modified_base 14..21: mod_base = OTHER; note = 2'-O-methyl nucleotide
  misc_feature 1..21: note = siRNA
caccttttcttctaatgagtt

SEQ ID NO: 18 - RNA, 23 nt, synthetic construct
  source 1..23: mol_type = other RNA
  modified_base 1: mod_base = OTHER; note = 2'-O-methyl nucleotide
  modified_base 1^2: mod_base = OTHER; note = Phosphorothioate Linkage
  modified_base 2: mod_base = OTHER; note = 2'-Fluoro nucleotide
  modified_base 2^3: mod_base = OTHER; note = Phosphorothioate Linkage
  modified_base 3..5: mod_base = OTHER; note = 2'-O-methyl nucleotide
  modified_base 6: mod_base = OTHER; note = 2'-Fluoro nucleotide
  modified_base 7..13: mod_base = OTHER; note = 2'-O-methyl nucleotide
  modified_base 14: mod_base = OTHER; note = 2'-Fluoro nucleotide
  modified_base 15: mod_base = OTHER; note = 2'-O-methyl nucleotide
  modified_base 16: mod_base = OTHER; note = 2'-Fluoro nucleotide
  modified_base 17..21: mod_base = OTHER; note = 2'-O-methyl nucleotide
  modified_base 21^22: mod_base = OTHER; note = Phosphorothioate Linkage
  modified_base 22: mod_base = OTHER; note = 2'-Fluoro nucleotide
  modified_base 22^23: mod_base = OTHER; note = Phosphorothioate Linkage
  modified_base 23: mod_base = OTHER; note = 2'-O-methyl nucleotide
  misc_feature 1..23: note = siRNA
aactcattagaagaaaaggtggg

SEQ ID NO: 19 - RNA, 21 nt, synthetic construct
  source 1..21: mol_type = other RNA
  modified_base 1..6: mod_base = OTHER; note = 2'-O-methyl nucleotide
  modified_base 1^2: mod_base = OTHER; note = Phosphorothioate Linkage
  modified_base 2^3: mod_base = OTHER; note = Phosphorothioate Linkage
  modified_base 7: mod_base = OTHER; note = 2'-Fluoro nucleotide
  modified_base 8: mod_base = OTHER; note = 2'-O-methyl nucleotide
  modified_base 9: mod_base = OTHER; note = 2'-Fluoro nucleotide
  modified_base 10: mod_base = OTHER; note = 2'-Fluoro nucleotide
  modified_base 11: mod_base = OTHER; note = 2'-Fluoro nucleotide
  modified_base 12: mod_base = OTHER; note = 2'-O-methyl nucleotide
  modified_base 13: mod_base = OTHER; note = 2'-Fluoro nucleotide
  modified_base 14..21: mod_base = OTHER; note = 2'-O-methyl nucleotide
  misc_feature 1..21: note = siRNA
gaccttttcttctaatgagtt

SEQ ID NO: 20 - RNA, 23 nt, synthetic construct
  source 1..23: mol_type = other RNA
  modified_base 1: mod_base = OTHER; note = 2'-O-methyl nucleotide
  modified_base 1^2: mod_base = OTHER; note = Phosphorothioate Linkage
  modified_base 2: mod_base = OTHER; note = 2'-Fluoro nucleotide
  modified_base 2^3: mod_base = OTHER; note = Phosphorothioate Linkage
  modified_base 3..5: mod_base = OTHER; note = 2'-O-methyl nucleotide
  modified_base 6: mod_base = OTHER; note = 2'-Fluoro nucleotide
  modified_base 7..13: mod_base = OTHER; note = 2'-O-methyl nucleotide
  modified_base 14: mod_base = OTHER; note = 2'-Fluoro nucleotide
  modified_base 15: mod_base = OTHER; note = 2'-O-methyl nucleotide
  modified_base 16: mod_base = OTHER; note = 2'-Fluoro nucleotide
  modified_base 17..21: mod_base = OTHER; note = 2'-O-methyl nucleotide
  modified_base 21^22: mod_base = OTHER; note = Phosphorothioate Linkage
  modified_base 22: mod_base = OTHER; note = 2'-Fluoro nucleotide
  modified_base 22^23: mod_base = OTHER; note = Phosphorothioate Linkage
  modified_base 23: mod_base = OTHER; note = 2'-O-methyl nucleotide
  misc_feature 1..23: note = siRNA
aactcattagaagaaaaggtcgg

SEQ ID NO: 21 - RNA, 21 nt, synthetic construct
  source 1..21: mol_type = other RNA
  modified_base 1..6: mod_base = OTHER; note = 2'-O-methyl nucleotide
  modified_base 1^2: mod_base = OTHER; note = Phosphorothioate Linkage
  modified_base 2^3: mod_base = OTHER; note = Phosphorothioate Linkage
  modified_base 7: mod_base = OTHER; note = 2'-Fluoro nucleotide
  modified_base 8: mod_base = OTHER; note = 2'-O-methyl nucleotide
  modified_base 9: mod_base = OTHER; note = 2'-Fluoro nucleotide
  modified_base 10: mod_base = OTHER; note = 2'-Fluoro nucleotide
  modified_base 11: mod_base = OTHER; note = 2'-Fluoro nucleotide
  modified_base 12: mod_base = OTHER; note = 2'-O-methyl nucleotide
  modified_base 13: mod_base = OTHER; note = 2'-Fluoro nucleotide
  modified_base 14..21: mod_base = OTHER; note = 2'-O-methyl nucleotide
  misc_feature 1..21: note = siRNA
ctccttttcttctaatgagtt

SEQ ID NO: 22 - RNA, 23 nt, synthetic construct
  source 1..23: mol_type = other RNA
  modified_base 1: mod_base = OTHER; note = 2'-O-methyl nucleotide
  modified_base 1^2: mod_base = OTHER; note = Phosphorothioate Linkage
  modified_base 2: mod_base = OTHER; note = 2'-Fluoro nucleotide
  modified_base 2^3: mod_base = OTHER; note = Phosphorothioate Linkage
  modified_base 3..5: mod_base = OTHER; note = 2'-O-methyl nucleotide
  modified_base 6: mod_base = OTHER; note = 2'-Fluoro nucleotide
  modified_base 7..13: mod_base = OTHER; note = 2'-O-methyl nucleotide
  modified_base 14: mod_base = OTHER; note = 2'-Fluoro nucleotide
  modified_base 15: mod_base = OTHER; note = 2'-O-methyl nucleotide
  modified_base 16: mod_base = OTHER; note = 2'-Fluoro nucleotide
  modified_base 17..21: mod_base = OTHER; note = 2'-O-methyl nucleotide
  modified_base 21^22: mod_base = OTHER; note = Phosphorothioate Linkage
  modified_base 22: mod_base = OTHER; note = 2'-Fluoro nucleotide
  modified_base 22^23: mod_base = OTHER; note = Phosphorothioate Linkage
  modified_base 23: mod_base = OTHER; note = 2'-O-methyl nucleotide
  misc_feature 1..23: note = siRNA
aactcattagaagaaaaggaggg

SEQ ID NO: 23 - RNA, 21 nt, synthetic construct
  source 1..21: mol_type = other RNA
  modified_base 1..6: mod_base = OTHER; note = 2'-O-methyl nucleotide
  modified_base 1^2: mod_base = OTHER; note = Phosphorothioate Linkage
  modified_base 2^3: mod_base = OTHER; note = Phosphorothioate Linkage
  modified_base 7: mod_base = OTHER; note = 2'-Fluoro nucleotide
  modified_base 8: mod_base = OTHER; note = 2'-O-methyl nucleotide
  modified_base 9: mod_base = OTHER; note = 2'-Fluoro nucleotide
  modified_base 10: mod_base = OTHER; note = 2'-Fluoro nucleotide
  modified_base 11: mod_base = OTHER; note = 2'-Fluoro nucleotide
  modified_base 12: mod_base = OTHER; note = 2'-O-methyl nucleotide
  modified_base 13: mod_base = OTHER; note = 2'-Fluoro nucleotide
  modified_base 14..21: mod_base = OTHER; note = 2'-O-methyl nucleotide
  misc_feature 1..21: note = siRNA
cagcttttcttctaatgagtt

SEQ ID NO: 24 - RNA, 23 nt, synthetic construct
  source 1..23: mol_type = other RNA
  modified_base 1: mod_base = OTHER; note = 2'-O-methyl nucleotide
  modified_base 1^2: mod_base = OTHER; note = Phosphorothioate Linkage
  modified_base 2: mod_base = OTHER; note = 2'-Fluoro nucleotide
  modified_base 2^3: mod_base = OTHER; note = Phosphorothioate Linkage
  modified_base 3..5: mod_base = OTHER; note = 2'-O-methyl nucleotide
  modified_base 6: mod_base = OTHER; note = 2'-Fluoro nucleotide
  modified_base 7..13: mod_base = OTHER; note = 2'-O-methyl nucleotide
  modified_base 14: mod_base = OTHER; note = 2'-Fluoro nucleotide
  modified_base 15: mod_base = OTHER; note = 2'-O-methyl nucleotide
  modified_base 16: mod_base = OTHER; note = 2'-Fluoro nucleotide
  modified_base 17..21: mod_base = OTHER; note = 2'-O-methyl nucleotide
  modified_base 21^22: mod_base = OTHER; note = Phosphorothioate Linkage
  modified_base 22: mod_base = OTHER; note = 2'-Fluoro nucleotide
  modified_base 22^23: mod_base = OTHER; note = Phosphorothioate Linkage
  modified_base 23: mod_base = OTHER; note = 2'-O-methyl nucleotide
  misc_feature 1..23: note = siRNA
aactcattagaagaaaagctggg

SEQ ID NO: 25 - RNA, 21 nt, synthetic construct
  source 1..21: mol_type = other RNA
  modified_base 1..6: mod_base = OTHER; note = 2'-O-methyl nucleotide
  modified_base 1^2: mod_base = OTHER; note = Phosphorothioate Linkage
  modified_base 2^3: mod_base = OTHER; note = Phosphorothioate Linkage
  modified_base 7: mod_base = OTHER; note = 2'-Fluoro nucleotide
  modified_base 8: mod_base = OTHER; note = 2'-O-methyl nucleotide
  modified_base 9: mod_base = OTHER; note = 2'-Fluoro nucleotide
  modified_base 10: mod_base = OTHER; note = 2'-Fluoro nucleotide
  modified_base 11: mod_base = OTHER; note = 2'-Fluoro nucleotide
  modified_base 12: mod_base = OTHER; note = 2'-O-methyl nucleotide
  modified_base 13: mod_base = OTHER; note = 2'-Fluoro nucleotide
  modified_base 14..16: mod_base = OTHER; note = 2'-O-methyl nucleotide
  modified_base 17: mod_base = OTHER; note = 2'-Fluoro nucleotide
  modified_base 18..21: mod_base = OTHER; note = 2'-O-methyl nucleotide
  modified_base 21: mod_base = OTHER; note = GalNAc(L96) modification
  misc_feature 1..21: note = siRNA
tcccaccttttcttctaatga

SEQ ID NO: 26 - RNA, 23 nt, synthetic construct
  source 1..23: mol_type = other RNA
  modified_base 1: mod_base = OTHER; note = 2'-O-methyl nucleotide
  modified_base 1^2: mod_base = OTHER; note = Phosphorothioate Linkage
  modified_base 2: mod_base = OTHER; note = 2'-Fluoro nucleotide
  modified_base 2^3: mod_base = OTHER; note = Phosphorothioate Linkage
  modified_base 3..5: mod_base = OTHER; note = 2'-O-methyl nucleotide
  modified_base 6: mod_base = OTHER; note = 2'-Fluoro nucleotide
  modified_base 7..13: mod_base = OTHER; note = 2'-O-methyl nucleotide
  modified_base 14: mod_base = OTHER; note = 2'-Fluoro nucleotide
  modified_base 15: mod_base = OTHER; note = 2'-O-methyl nucleotide
  modified_base 16: mod_base = OTHER; note = 2'-Fluoro nucleotide
  modified_base 17..21: mod_base = OTHER; note = 2'-O-methyl nucleotide
  modified_base 21^22: mod_base = OTHER; note = Phosphorothioate Linkage
  modified_base 22: mod_base = OTHER; note = 2'-Fluoro nucleotide
  modified_base 22^23: mod_base = OTHER; note = Phosphorothioate Linkage
  modified_base 23: mod_base = OTHER; note = 2'-O-methyl nucleotide
  misc_feature 1..23: note = siRNA
tcattagaagaaaaggtgggaga

SEQ ID NO: 27 - RNA, 21 nt, synthetic construct
  source 1..21: mol_type = other RNA
  modified_base 1..6: mod_base = OTHER; note = 2'-O-methyl nucleotide
  modified_base 1^2: mod_base = OTHER; note = Phosphorothioate Linkage
  modified_base 2^3: mod_base = OTHER; note = Phosphorothioate Linkage
  modified_base 7: mod_base = OTHER; note = 2'-Fluoro nucleotide
  modified_base 8: mod_base = OTHER; note = 2'-O-methyl nucleotide
  modified_base 9: mod_base = OTHER; note = 2'-Fluoro nucleotide
  modified_base 10: mod_base = OTHER; note = 2'-Fluoro nucleotide
  modified_base 11: mod_base = OTHER; note = 2'-Fluoro nucleotide
  modified_base 12: mod_base = OTHER; note = 2'-O-methyl nucleotide
  modified_base 13: mod_base = OTHER; note = 2'-Fluoro nucleotide
  modified_base 14..16: mod_base = OTHER; note = 2'-O-methyl nucleotide
  modified_base 17: mod_base = OTHER; note = 2'-Fluoro nucleotide
  modified_base 18..21: mod_base = OTHER; note = 2'-O-methyl nucleotide
  modified_base 21: mod_base = OTHER; note = GalNAc(L96) modification
  misc_feature 1..21: note = siRNA
acccaccttttcttctaatga

SEQ ID NO: 28 - RNA, 23 nt, synthetic construct
  source 1..23: mol_type = other RNA
  modified_base 1: mod_base = OTHER; note = 2'-O-methyl nucleotide
  modified_base 1^2: mod_base = OTHER; note = Phosphorothioate Linkage
  modified_base 2: mod_base = OTHER; note = 2'-Fluoro nucleotide
  modified_base 2^3: mod_base = OTHER; note = Phosphorothioate Linkage
  modified_base 3..5: mod_base = OTHER; note = 2'-O-methyl nucleotide
  modified_base 6: mod_base = OTHER; note = 2'-Fluoro nucleotide
  modified_base 7..13: mod_base = OTHER; note = 2'-O-methyl nucleotide
  modified_base 14: mod_base = OTHER; note = 2'-Fluoro nucleotide
  modified_base 15: mod_base = OTHER; note = 2'-O-methyl nucleotide
  modified_base 16: mod_base = OTHER; note = 2'-Fluoro nucleotide
  modified_base 17..21: mod_base = OTHER; note = 2'-O-methyl nucleotide
  modified_base 21^22: mod_base = OTHER; note = Phosphorothioate Linkage
  modified_base 22: mod_base = OTHER; note = 2'-Fluoro nucleotide
  modified_base 22^23: mod_base = OTHER; note = Phosphorothioate Linkage
  modified_base 23: mod_base = OTHER; note = 2'-O-methyl nucleotide
  misc_feature 1..23: note = siRNA
tcattagaagaaaaggtgggtga

SEQ ID NO: 29 - RNA, 21 nt, synthetic construct
  source 1..21: mol_type = other RNA
  modified_base 1..6: mod_base = OTHER; note = 2'-O-methyl nucleotide
  modified_base 1^2: mod_base = OTHER; note = Phosphorothioate Linkage
  modified_base 2^3: mod_base = OTHER; note = Phosphorothioate Linkage
  modified_base 7: mod_base = OTHER; note = 2'-Fluoro nucleotide
  modified_base 8: mod_base = OTHER; note = 2'-O-methyl nucleotide
  modified_base 9: mod_base = OTHER; note = 2'-Fluoro nucleotide
  modified_base 10: mod_base = OTHER; note = 2'-Fluoro nucleotide
  modified_base 11: mod_base = OTHER; note = 2'-Fluoro nucleotide
  modified_base 12: mod_base = OTHER; note = 2'-O-methyl nucleotide
  modified_base 13: mod_base = OTHER; note = 2'-Fluoro nucleotide
  modified_base 14..16: mod_base = OTHER; note = 2'-O-methyl nucleotide
  modified_base 17: mod_base = OTHER; note = 2'-Fluoro nucleotide
  modified_base 18..21: mod_base = OTHER; note = 2'-O-methyl nucleotide
  modified_base 21: mod_base = OTHER; note = GalNAc(L96) modification
  misc_feature 1..21: note = siRNA
tgccaccttttcttctaatga

SEQ ID NO: 30 - RNA, 23 nt, synthetic construct
  source 1..23: mol_type = other RNA
  modified_base 1: mod_base = OTHER; note = 2'-O-methyl nucleotide
  modified_base 1^2: mod_base = OTHER; note = Phosphorothioate Linkage
  modified_base 2: mod_base = OTHER; note = 2'-Fluoro nucleotide
  modified_base 2^3: mod_base = OTHER; note = Phosphorothioate Linkage
  modified_base 3..5: mod_base = OTHER; note = 2'-O-methyl nucleotide
  modified_base 6: mod_base = OTHER; note = 2'-Fluoro nucleotide
  modified_base 7..13: mod_base = OTHER; note = 2'-O-methyl nucleotide
  modified_base 14: mod_base = OTHER; note = 2'-Fluoro nucleotide
  modified_base 15: mod_base = OTHER; note = 2'-O-methyl nucleotide
  modified_base 16: mod_base = OTHER; note = 2'-Fluoro nucleotide
  modified_base 17..21: mod_base = OTHER; note = 2'-O-methyl nucleotide
  modified_base 21^22: mod_base = OTHER; note = Phosphorothioate Linkage
  modified_base 22: mod_base = OTHER; note = 2'-Fluoro nucleotide
  modified_base 22^23: mod_base = OTHER; note = Phosphorothioate Linkage
  modified_base 23: mod_base = OTHER; note = 2'-O-methyl nucleotide
  misc_feature 1..23: note = siRNA
tcattagaagaaaaggtggcaga

SEQ ID NO: 31 - RNA, 21 nt, synthetic construct
  source 1..21: mol_type = other RNA
  modified_base 1..6: mod_base = OTHER; note = 2'-O-methyl nucleotide
  modified_base 1^2: mod_base = OTHER; note = Phosphorothioate Linkage
  modified_base 2^3: mod_base = OTHER; note = Phosphorothioate Linkage
  modified_base 7: mod_base = OTHER; note = 2'-Fluoro nucleotide
  modified_base 8: mod_base = OTHER; note = 2'-O-methyl nucleotide
  modified_base 9: mod_base = OTHER; note = 2'-Fluoro nucleotide
  modified_base 10: mod_base = OTHER; note = 2'-Fluoro nucleotide
  modified_base 11: mod_base = OTHER; note = 2'-Fluoro nucleotide
  modified_base 12: mod_base = OTHER; note = 2'-O-methyl nucleotide
  modified_base 13: mod_base = OTHER; note = 2'-Fluoro nucleotide
  modified_base 14..16: mod_base = OTHER; note = 2'-O-methyl nucleotide
  modified_base 17: mod_base = OTHER; note = 2'-Fluoro nucleotide
  modified_base 18..21: mod_base = OTHER; note = 2'-O-methyl nucleotide
  modified_base 21: mod_base = OTHER; note = GalNAc(L96) modification
  misc_feature 1..21: note = siRNA
tcgcaccttttcttctaatga

SEQ ID NO: 32 - RNA, 23 nt, synthetic construct
  source 1..23: mol_type = other RNA
  modified_base 1: mod_base = OTHER; note = 2'-O-methyl nucleotide
  modified_base 1^2: mod_base = OTHER; note = Phosphorothioate Linkage
  modified_base 2: mod_base = OTHER; note = 2'-Fluoro nucleotide
  modified_base 2^3: mod_base = OTHER; note = Phosphorothioate Linkage
  modified_base 3..5: mod_base = OTHER; note = 2'-O-methyl nucleotide
  modified_base 6: mod_base = OTHER; note = 2'-Fluoro nucleotide
  modified_base 7..13: mod_base = OTHER; note = 2'-O-methyl nucleotide
  modified_base 14: mod_base = OTHER; note = 2'-Fluoro nucleotide
  modified_base 15: mod_base = OTHER; note = 2'-O-methyl nucleotide
  modified_base 16: mod_base = OTHER; note = 2'-Fluoro nucleotide
  modified_base 17..21: mod_base = OTHER; note = 2'-O-methyl nucleotide
  modified_base 21^22: mod_base = OTHER; note = Phosphorothioate Linkage
  modified_base 22: mod_base = OTHER; note = 2'-Fluoro nucleotide
  modified_base 22^23: mod_base = OTHER; note = Phosphorothioate Linkage
  modified_base 23: mod_base = OTHER; note = 2'-O-methyl nucleotide
  misc_feature 1..23: note = siRNA
tcattagaagaaaaggtgcgaga

SEQ ID NO: 33 - RNA, 21 nt, synthetic construct
  source 1..21: mol_type = other RNA
  modified_base 1..6: mod_base = OTHER; note = 2'-O-methyl nucleotide
  modified_base 1^2: mod_base = OTHER; note = Phosphorothioate Linkage
  modified_base 2^3: mod_base = OTHER; note = Phosphorothioate Linkage
  modified_base 7: mod_base = OTHER; note = 2'-Fluoro nucleotide
  modified_base 8: mod_base = OTHER; note = 2'-O-methyl nucleotide
  modified_base 9: mod_base = OTHER; note = 2'-Fluoro nucleotide
  modified_base 10: mod_base = OTHER; note = 2'-Fluoro nucleotide
  modified_base 11: mod_base = OTHER; note = 2'-Fluoro nucleotide
  modified_base 12: mod_base = OTHER; note = 2'-O-methyl nucleotide
  modified_base 13: mod_base = OTHER; note = 2'-Fluoro nucleotide
  modified_base 14..21: mod_base = OTHER; note = 2'-O-methyl nucleotide
  misc_feature 1..21: note = siRNA
ccccacaatgatgattaaaca

SEQ ID NO: 34 - RNA, 23 nt, synthetic construct
  source 1..23: mol_type = other RNA
  modified_base 1: mod_base = OTHER; note = (E)-vinyl phosphonate-modified nucleotide
  modified_base 1: mod_base = OTHER; note = 2'-O-methyl nucleotide
  modified_base 1^2: mod_base = OTHER; note = Phosphorothioate Linkage
  modified_base 2: mod_base = OTHER; note = 2'-Fluoro nucleotide
  modified_base 2^3: mod_base = OTHER; note = Phosphorothioate Linkage
  modified_base 3..5: mod_base = OTHER; note = 2'-O-methyl nucleotide
  modified_base 6: mod_base = OTHER; note = 2'-Fluoro nucleotide
  modified_base 7..13: mod_base = OTHER; note = 2'-O-methyl nucleotide
  modified_base 14: mod_base = OTHER; note = 2'-Fluoro nucleotide
  modified_base 15: mod_base = OTHER; note = 2'-O-methyl nucleotide
  modified_base 16: mod_base = OTHER; note = 2'-Fluoro nucleotide
  modified_base 17..21: mod_base = OTHER; note = 2'-O-methyl nucleotide
  modified_base 21^22: mod_base = OTHER; note = Phosphorothioate Linkage
  modified_base 22: mod_base = OTHER; note = 2'-Fluoro nucleotide
  modified_base 22^23: mod_base = OTHER; note = Phosphorothioate Linkage
  modified_base 23: mod_base = OTHER; note = 2'-O-methyl nucleotide
  misc_feature 1..23: note = siRNA
tgtttaatcatcattgtgggggg

SEQ ID NO: 35 - RNA, 21 nt, synthetic construct
  source 1..21: mol_type = other RNA
  modified_base 1..6: mod_base = OTHER; note = 2'-O-methyl nucleotide
  modified_base 1^2: mod_base = OTHER; note = Phosphorothioate Linkage
  modified_base 2^3: mod_base = OTHER; note = Phosphorothioate Linkage
  modified_base 7: mod_base = OTHER; note = 2'-Fluoro nucleotide
  modified_base 8: mod_base = OTHER; note = 2'-O-methyl nucleotide
  modified_base 9: mod_base = OTHER; note = 2'-Fluoro nucleotide
  modified_base 10: mod_base = OTHER; note = 2'-Fluoro nucleotide
  modified_base 11: mod_base = OTHER; note = 2'-Fluoro nucleotide
  modified_base 12: mod_base = OTHER; note = 2'-O-methyl nucleotide
  modified_base 13: mod_base = OTHER; note = 2'-Fluoro nucleotide
  modified_base 14..21: mod_base = OTHER; note = 2'-O-methyl nucleotide
  misc_feature 1..21: note = siRNA
gcccacaatgatgattaaaca

SEQ ID NO: 36 - RNA, 23 nt, synthetic construct
  source 1..23: mol_type = other RNA
  modified_base 1: mod_base = OTHER; note = (E)-vinyl phosphonate-modified nucleotide
  modified_base 1: mod_base = OTHER; note = 2'-O-methyl nucleotide
  modified_base 1^2: mod_base = OTHER; note = Phosphorothioate Linkage
  modified_base 2: mod_base = OTHER; note = 2'-Fluoro nucleotide
  modified_base 2^3: mod_base = OTHER; note = Phosphorothioate Linkage
  modified_base 3..5: mod_base = OTHER; note = 2'-O-methyl nucleotide
  modified_base 6: mod_base = OTHER; note = 2'-Fluoro nucleotide
  modified_base 7..13: mod_base = OTHER; note = 2'-O-methyl nucleotide
  modified_base 14: mod_base = OTHER; note = 2'-Fluoro nucleotide
  modified_base 15: mod_base = OTHER; note = 2'-O-methyl nucleotide
  modified_base 16: mod_base = OTHER; note = 2'-Fluoro nucleotide
  modified_base 17..21: mod_base = OTHER; note = 2'-O-methyl nucleotide
  modified_base 21^22: mod_base = OTHER; note = Phosphorothioate Linkage
  modified_base 22: mod_base = OTHER; note = 2'-Fluoro nucleotide
  modified_base 22^23: mod_base = OTHER; note = Phosphorothioate Linkage
  modified_base 23: mod_base = OTHER; note = 2'-O-methyl nucleotide
  misc_feature 1..23: note = siRNA
tgtttaatcatcattgtgggcgg

SEQ ID NO: 37 - RNA, 21 nt, synthetic construct
  source 1..21: mol_type = other RNA
  modified_base 1..6: mod_base = OTHER; note = 2'-O-methyl nucleotide
  modified_base 1^2: mod_base = OTHER; note = Phosphorothioate Linkage
  modified_base 2^3: mod_base = OTHER; note = Phosphorothioate Linkage
  modified_base 7: mod_base = OTHER; note = 2'-Fluoro nucleotide
  modified_base 8: mod_base = OTHER; note = 2'-O-methyl nucleotide
  modified_base 9: mod_base = OTHER; note = 2'-Fluoro nucleotide
  modified_base 10: mod_base = OTHER; note = 2'-Fluoro nucleotide
  modified_base 11: mod_base = OTHER; note = 2'-Fluoro nucleotide
  modified_base 12: mod_base = OTHER; note = 2'-O-methyl nucleotide
  modified_base 13: mod_base = OTHER; note = 2'-Fluoro nucleotide
  modified_base 14..21: mod_base = OTHER; note = 2'-O-methyl nucleotide
  misc_feature 1..21: note = siRNA
cgccacaatgatgattaaaca

SEQ ID NO: 38 - RNA, 23 nt, synthetic construct
  source 1..23: mol_type = other RNA
  modified_base 1: mod_base = OTHER; note = (E)-vinyl phosphonate-modified nucleotide
  modified_base 1: mod_base = OTHER; note = 2'-O-methyl nucleotide
  modified_base 1^2: mod_base = OTHER; note = Phosphorothioate Linkage
  modified_base 2: mod_base = OTHER; note = 2'-Fluoro nucleotide
  modified_base 2^3: mod_base = OTHER; note = Phosphorothioate Linkage
  modified_base 3..5: mod_base = OTHER; note = 2'-O-methyl nucleotide
  modified_base 6: mod_base = OTHER; note = 2'-Fluoro nucleotide
  modified_base 7..13: mod_base = OTHER; note = 2'-O-methyl nucleotide
  modified_base 14: mod_base = OTHER; note = 2'-Fluoro nucleotide
  modified_base 15: mod_base = OTHER; note = 2'-O-methyl nucleotide
  modified_base 16: mod_base = OTHER; note = 2'-Fluoro nucleotide
  modified_base 17..21: mod_base = OTHER; note = 2'-O-methyl nucleotide
  modified_base 21^22: mod_base = OTHER; note = Phosphorothioate Linkage
  modified_base 22: mod_base = OTHER; note = 2'-Fluoro nucleotide
  modified_base 22^23: mod_base = OTHER; note = Phosphorothioate Linkage
  modified_base 23: mod_base = OTHER; note = 2'-O-methyl nucleotide
  misc_feature 1..23: note = siRNA
tgtttaatcatcattgtggcggg

SEQ ID NO: 39 - RNA, 21 nt, synthetic construct
  source 1..21: mol_type = other RNA
  modified_base 1..6: mod_base = OTHER; note = 2'-O-methyl nucleotide
  modified_base 1^2: mod_base = OTHER; note = Phosphorothioate Linkage
  modified_base 2^3: mod_base = OTHER; note = Phosphorothioate Linkage
  modified_base 7: mod_base = OTHER; note = 2'-Fluoro nucleotide
  modified_base 8: mod_base = OTHER; note = 2'-O-methyl nucleotide
  modified_base 9: mod_base = OTHER; note = 2'-Fluoro nucleotide
  modified_base 10: mod_base = OTHER; note = 2'-Fluoro nucleotide
  modified_base 11: mod_base = OTHER; note = 2'-Fluoro nucleotide
  modified_base 12: mod_base = OTHER; note = 2'-O-methyl nucleotide
  modified_base 13: mod_base = OTHER; note = 2'-Fluoro nucleotide
  modified_base 14..21: mod_base = OTHER; note = 2'-O-methyl nucleotide
  misc_feature 1..21: note = siRNA
ccgcacaatgatgattaaaca

SEQ ID NO: 40 - RNA, 23 nt, synthetic construct
  source 1..23: mol_type = other RNA
  modified_base 1: mod_base = OTHER; note = (E)-vinyl phosphonate-modified nucleotide
  modified_base 1: mod_base = OTHER; note = 2'-O-methyl nucleotide
  modified_base 1^2: mod_base = OTHER; note = Phosphorothioate Linkage
  modified_base 2: mod_base = OTHER; note = 2'-Fluoro nucleotide
  modified_base 2^3: mod_base = OTHER; note = Phosphorothioate Linkage
  modified_base 3..5: mod_base = OTHER; note = 2'-O-methyl nucleotide
  modified_base 6: mod_base = OTHER; note = 2'-Fluoro nucleotide
  modified_base 7..13: mod_base = OTHER; note = 2'-O-methyl nucleotide
  modified_base 14: mod_base = OTHER; note = 2'-Fluoro nucleotide
  modified_base 15: mod_base = OTHER; note = 2'-O-methyl nucleotide
  modified_base 16: mod_base = OTHER; note = 2'-Fluoro nucleotide
  modified_base 17..21: mod_base = OTHER; note = 2'-O-methyl nucleotide
  modified_base 21^22: mod_base = OTHER; note = Phosphorothioate Linkage
  modified_base 22: mod_base = OTHER; note = 2'-Fluoro nucleotide
  modified_base 22^23: mod_base = OTHER; note = Phosphorothioate Linkage
  modified_base 23: mod_base = OTHER; note = 2'-O-methyl nucleotide
  misc_feature 1..23: note = siRNA
tgtttaatcatcattgtgcgggg

SEQ ID NO: 41 - RNA, 21 nt, synthetic construct
  source 1..21: mol_type = other RNA
  modified_base 1..6: mod_base = OTHER; note = 2'-O-methyl nucleotide
  modified_base 1^2: mod_base = OTHER; note = Phosphorothioate Linkage
  modified_base 2^3: mod_base = OTHER; note = Phosphorothioate Linkage
  modified_base 7: mod_base = OTHER; note = 2'-Fluoro nucleotide
  modified_base 8: mod_base = OTHER; note = 2'-O-methyl nucleotide
  modified_base 9: mod_base = OTHER; note = 2'-Fluoro nucleotide
  modified_base 10: mod_base = OTHER; note = 2'-Fluoro nucleotide
  modified_base 11: mod_base = OTHER; note = 2'-Fluoro nucleotide
  modified_base 12: mod_base = OTHER; note = 2'-O-methyl nucleotide
  modified_base 13: mod_base = OTHER; note = 2'-Fluoro nucleotide
  modified_base 14..21: mod_base = OTHER; note = 2'-O-methyl nucleotide
  modified_base 21: mod_base = OTHER; note = GalNAc(L96) modification
  misc_feature 1..21: note = siRNA
caccttttcttctaatgagta

SEQ ID NO: 42 - RNA, 23 nt, synthetic construct
  source 1..23: mol_type = other RNA
  modified_base 1: mod_base = OTHER; note = (E)-vinyl phosphonate-modified nucleotide
  modified_base 1: mod_base = OTHER; note = 2'-O-methyl nucleotide
  modified_base 1^2: mod_base = OTHER; note = Phosphorothioate Linkage
  modified_base 2: mod_base = OTHER; note = 2'-Fluoro nucleotide
  modified_base 2^3: mod_base = OTHER; note = Phosphorothioate Linkage
  modified_base 3..5: mod_base = OTHER; note = 2'-O-methyl nucleotide
  modified_base 6: mod_base = OTHER; note = 2'-Fluoro nucleotide
  modified_base 7..13: mod_base = OTHER; note = 2'-O-methyl nucleotide
  modified_base 14: mod_base = OTHER; note = 2'-Fluoro nucleotide
  modified_base 15: mod_base = OTHER; note = 2'-O-methyl nucleotide
  modified_base 16: mod_base = OTHER; note = 2'-Fluoro nucleotide
  modified_base 17..21: mod_base = OTHER; note = 2'-O-methyl nucleotide
  modified_base 21^22: mod_base = OTHER; note = Phosphorothioate Linkage
  modified_base 22: mod_base = OTHER; note = 2'-Fluoro nucleotide
  modified_base 22^23: mod_base = OTHER; note = Phosphorothioate Linkage
  modified_base 23: mod_base = OTHER; note = 2'-O-methyl nucleotide
  misc_feature 1..23: note = siRNA
tactcattagaagaaaaggtggg

SEQ ID NO: 43 - RNA, 21 nt, synthetic construct
  source 1..21: mol_type = other RNA
  modified_base 1..6: mod_base = OTHER; note = 2'-O-methyl nucleotide
  modified_base 1^2: mod_base = OTHER; note = Phosphorothioate Linkage
  modified_base 2^3: mod_base = OTHER; note = Phosphorothioate Linkage
  modified_base 7: mod_base = OTHER; note = 2'-Fluoro nucleotide
  modified_base 8: mod_base = OTHER; note = 2'-O-methyl nucleotide
  modified_base 9: mod_base = OTHER; note = 2'-Fluoro nucleotide
  modified_base 10: mod_base = OTHER; note = 2'-Fluoro nucleotide
  modified_base 11: mod_base = OTHER; note = 2'-Fluoro nucleotide
  modified_base 12: mod_base = OTHER; note = 2'-O-methyl nucleotide
  modified_base 13: mod_base = OTHER; note = 2'-Fluoro nucleotide
  modified_base 14..21: mod_base = OTHER; note = 2'-O-methyl nucleotide
  modified_base 21: mod_base = OTHER; note = GalNAc(L96) modification
  misc_feature 1..21: note = siRNA
ctccttttcttctaatgagta

SEQ ID NO: 44 - RNA, 23 nt, synthetic construct
  source 1..23: mol_type = other RNA
  modified_base 1: mod_base = OTHER; note = (E)-vinyl phosphonate-modified nucleotide
  modified_base 1: mod_base = OTHER; note = 2'-O-methyl nucleotide
  modified_base 1^2: mod_base = OTHER; note = Phosphorothioate Linkage
  modified_base 2: mod_base = OTHER; note = 2'-Fluoro nucleotide
  modified_base 2^3: mod_base = OTHER; note = Phosphorothioate Linkage
  modified_base 3..5: mod_base = OTHER; note = 2'-O-methyl nucleotide
  modified_base 6: mod_base = OTHER; note = 2'-Fluoro nucleotide
  modified_base 7..13: mod_base = OTHER; note = 2'-O-methyl nucleotide
  modified_base 14: mod_base = OTHER; note = 2'-Fluoro nucleotide
  modified_base 15: mod_base = OTHER; note = 2'-O-methyl nucleotide
  modified_base 16: mod_base = OTHER; note = 2'-Fluoro nucleotide
  modified_base 17..21: mod_base = OTHER; note = 2'-O-methyl nucleotide
  modified_base 21^22: mod_base = OTHER; note = Phosphorothioate Linkage
  modified_base 22: mod_base = OTHER; note = 2'-Fluoro nucleotide
  modified_base 22^23: mod_base = OTHER; note = Phosphorothioate Linkage
  modified_base 23: mod_base = OTHER; note = 2'-O-methyl nucleotide
  misc_feature 1..23: note = siRNA
tactcattagaagaaaaggaggg

SEQ ID NO: 45 - RNA, 23 nt, synthetic construct
  source 1..23: mol_type = other RNA
  modified_base 1: mod_base = OTHER; note = (E)-vinyl phosphonate-modified nucleotide
  modified_base 1: mod_base = OTHER; note = 2'-O-methyl nucleotide
  modified_base 1^2: mod_base = OTHER; note = Phosphorothioate Linkage
  modified_base 2: mod_base = OTHER; note = 2'-Fluoro nucleotide
  modified_base 2^3: mod_base = OTHER; note = Phosphorothioate Linkage
  modified_base 3..5: mod_base = OTHER; note = 2'-O-methyl nucleotide
  modified_base 6: mod_base = OTHER; note = 2'-Fluoro nucleotide
  modified_base 7: mod_base = OTHER; note = 2'-Fluoro nucleotide
  modified_base 8..13: mod_base = OTHER; note = 2'-O-methyl nucleotide
  modified_base 14: mod_base = OTHER; note = 2'-Fluoro nucleotide
  modified_base 15: mod_base = OTHER; note = 2'-O-methyl nucleotide
  modified_base 16: mod_base = OTHER; note = 2'-Fluoro nucleotide
  modified_base 17..21: mod_base = OTHER; note = 2'-O-methyl nucleotide
  modified_base 21^22: mod_base = OTHER; note = Phosphorothioate Linkage
  modified_base 22: mod_base = OTHER; note = 2'-Fluoro nucleotide
  modified_base 22^23: mod_base = OTHER; note = Phosphorothioate Linkage
  modified_base 23: mod_base = OTHER; note = 2'-O-methyl nucleotide
  misc_feature 1..23: note = siRNA
tactcattagaagaaaaggtggg

SEQ ID NO: 46 - RNA, 23 nt, synthetic construct
  source 1..23: mol_type = other RNA
  modified_base 1: mod_base = OTHER; note = (E)-vinyl phosphonate-modified nucleotide
  modified_base 1: mod_base = OTHER; note = 2'-O-methyl nucleotide
  modified_base 1^2: mod_base = OTHER; note = Phosphorothioate Linkage
  modified_base 2: mod_base = OTHER; note = 2'-Fluoro nucleotide
  modified_base 2^3: mod_base = OTHER; note = Phosphorothioate Linkage
  modified_base 3..5: mod_base = OTHER; note = 2'-O-methyl nucleotide
  modified_base 6: mod_base = OTHER; note = 2'-Fluoro nucleotide
  modified_base 7: mod_base = OTHER; note = 2'-Fluoro nucleotide
  modified_base 8..13: mod_base = OTHER; note = 2'-O-methyl nucleotide
  modified_base 14: mod_base = OTHER; note = 2'-Fluoro nucleotide
  modified_base 15: mod_base = OTHER; note = 2'-O-methyl nucleotide
  modified_base 16: mod_base = OTHER; note = 2'-Fluoro nucleotide
  modified_base 17..21: mod_base = OTHER; note = 2'-O-methyl nucleotide
  modified_base 21^22: mod_base = OTHER; note = Phosphorothioate Linkage
  modified_base 22: mod_base = OTHER; note = 2'-Fluoro nucleotide
  modified_base 22^23: mod_base = OTHER; note = Phosphorothioate Linkage
  modified_base 23: mod_base = OTHER; note = 2'-O-methyl nucleotide
  misc_feature 1..23: note = siRNA
tactcattagaagaaaaggaggg

SEQ ID NO: 47 - RNA, 21 nt, synthetic construct
  source 1..21: mol_type = other RNA
  modified_base 1..6: mod_base = OTHER; note = 2'-O-methyl nucleotide
  modified_base 1^2: mod_base = OTHER; note = Phosphorothioate Linkage
  modified_base 2^3: mod_base = OTHER; note = Phosphorothioate Linkage
  modified_base 7: mod_base = OTHER; note = 2'-Fluoro nucleotide
  modified_base 8: mod_base = OTHER; note = 2'-O-methyl nucleotide
  modified_base 9: mod_base = OTHER; note = 2'-Fluoro nucleotide
  modified_base 10: mod_base = OTHER; note = 2'-Fluoro nucleotide
  modified_base 11: mod_base = OTHER; note = 2'-Fluoro nucleotide
  modified_base 12..21: mod_base = OTHER; note = 2'-O-methyl nucleotide
  misc_feature 1..21: note = siRNA
gtcatccacaatgagagtaca

SEQ ID NO: 48 - RNA, 23 nt, synthetic construct
  source 1..23: mol_type = other RNA
  modified_base 1: mod_base = OTHER; note = 2'-O-methyl nucleotide
  modified_base 1^2: mod_base = OTHER; note = Phosphorothioate Linkage
  modified_base 2: mod_base = OTHER; note = 2'-Fluoro nucleotide
  modified_base 2^3: mod_base = OTHER; note = Phosphorothioate Linkage
  modified_base 3..5: mod_base = OTHER; note = 2'-O-methyl nucleotide
  modified_base 6: mod_base = OTHER; note = Thymine
  modified_base 7..13: mod_base = OTHER; note = 2'-O-methyl nucleotide
  modified_base 14: mod_base = OTHER; note = 2'-Fluoro nucleotide
  modified_base 15: mod_base = OTHER; note = 2'-O-methyl nucleotide
  modified_base 16: mod_base = OTHER; note = 2'-Fluoro nucleotide
  modified_base 17..23: mod_base = OTHER; note = 2'-O-methyl nucleotide
  modified_base 21^22: mod_base = OTHER; note = Phosphorothioate Linkage
  modified_base 22^23: mod_base = OTHER; note = Phosphorothioate Linkage
  misc_feature 1..23: note = siRNA
  modified_base 6: mod_base = OTHER; note = GNA
tgtactctcattgtggatgacga

SEQ ID NO: 49 - RNA, 21 nt, synthetic construct
  source 1..21: mol_type = other RNA
  modified_base 1..6: mod_base = OTHER; note = 2'-O-methyl nucleotide
  modified_base 1^2: mod_base = OTHER; note = Phosphorothioate Linkage
  modified_base 2^3: mod_base = OTHER; note = Phosphorothioate Linkage
  modified_base 7: mod_base = OTHER; note = 2'-Fluoro nucleotide
  modified_base 8: mod_base = OTHER; note = 2'-O-methyl nucleotide
  modified_base 9: mod_base = OTHER; note = 2'-Fluoro nucleotide
  modified_base 10: mod_base = OTHER; note = 2'-Fluoro nucleotide
  modified_base 11: mod_base = OTHER; note = 2'-Fluoro nucleotide
  modified_base 12..21: mod_base = OTHER; note = 2'-O-methyl nucleotide
  modified_base 21: mod_base = OTHER; note = GalNAc(L96) modification
  misc_feature 1..21: note = siRNA
gtcatccacaatgagagtaca

SEQ ID NO: 50 - RNA, 23 nt, synthetic construct
  source 1..23: mol_type = other RNA
  modified_base 1: mod_base = OTHER; note = 2'-O-methyl nucleotide
  modified_base 1^2: mod_base = OTHER; note = Phosphorothioate Linkage
  modified_base 2: mod_base = OTHER; note = 2'-Fluoro nucleotide
  modified_base 2^3: mod_base = OTHER; note = Phosphorothioate Linkage
  modified_base 3..5: mod_base = OTHER; note = 2'-O-methyl nucleotide
  modified_base 6: mod_base = OTHER; note = Thymine
  modified_base 7..13: mod_base = OTHER; note = 2'-O-methyl nucleotide
  modified_base 14: mod_base = OTHER; note = 2'-Fluoro nucleotide
  modified_base 15: mod_base = OTHER; note = 2'-O-methyl nucleotide
  modified_base 16: mod_base = OTHER; note = 2'-Fluoro nucleotide
  modified_base 17..23: mod_base = OTHER; note = 2'-O-methyl nucleotide
  modified_base 21^22: mod_base = OTHER; note = Phosphorothioate Linkage
  modified_base 22^23: mod_base = OTHER; note = Phosphorothioate Linkage
  misc_feature 1..23: note = siRNA
  modified_base 6: mod_base = OTHER; note = GNA
tgtactctcattgtggatgacga

SEQ ID NO: 51 - RNA, 21 nt, synthetic construct
  source 1..21: mol_type = other RNA
  modified_base 1: mod_base = OTHER; note = invAb is linked to nucleotide through phosphorothioate group
  modified_base 1..8: mod_base = OTHER; note = 2'-O-methyl nucleotide
  modified_base 9: mod_base = OTHER; note = 2'-Fluoro nucleotide
  modified_base 10: mod_base = OTHER; note = 2'-Fluoro nucleotide
  modified_base 11: mod_base = OTHER; note = 2'-Fluoro nucleotide
  modified_base 12..21: mod_base = OTHER; note = 2'-O-methyl nucleotide
  modified_base 21: mod_base = OTHER; note = invAb is linked to nucleotide through phosphorothioate group
  misc_feature 1..21: note = siRNA
tagtaggtgctcaaaacatca

SEQ ID NO: 52 - RNA, 21 nt, synthetic construct
  source 1..21: mol_type = other RNA
  modified_base 1: mod_base = OTHER; note = (E)-vinyl phosphonate-modified nucleotide
  modified_base 1: mod_base = OTHER; note = 2'-O-methyl nucleotide
  modified_base 1^2: mod_base = OTHER; note = Phosphorothioate Linkage
  modified_base 2: mod_base = OTHER; note = 2'-Fluoro nucleotide
  modified_base 2^3: mod_base = OTHER; note = Phosphorothioate Linkage
  modified_base 3: mod_base = OTHER; note = 2'-O-methyl nucleotide
  modified_base 3^4: mod_base = OTHER; note = Phosphorothioate Linkage
  modified_base 4: mod_base = OTHER; note = 2'-Fluoro nucleotide
  modified_base 5: mod_base = OTHER; note = 2'-O-methyl nucleotide
  modified_base 6: mod_base = OTHER; note = 2'-Fluoro nucleotide
  modified_base 7: mod_base = OTHER; note = 2'-O-methyl nucleotide
  modified_base 8: mod_base = OTHER; note = 2'-Fluoro nucleotide
  modified_base 9: mod_base = OTHER; note = 2'-O-methyl nucleotide
  modified_base 10: mod_base = OTHER; note = 2'-Fluoro nucleotide
  modified_base 11: mod_base = OTHER; note = 2'-O-methyl nucleotide
  modified_base 12: mod_base = OTHER; note = 2'-Fluoro nucleotide
  modified_base 13: mod_base = OTHER; note = 2'-O-methyl nucleotide
  modified_base 14: mod_base = OTHER; note = 2'-Fluoro nucleotide
  modified_base 15: mod_base = OTHER; note = 2'-O-methyl nucleotide
  modified_base 16: mod_base = OTHER; note = 2'-Fluoro nucleotide
  modified_base 17: mod_base = OTHER; note = 2'-O-methyl nucleotide
  modified_base 18: mod_base = OTHER; note = 2'-Fluoro nucleotide
  modified_base 19: mod_base = OTHER; note = 2'-O-methyl nucleotide
  modified_base 20: mod_base = OTHER; note = 2'-Fluoro nucleotide
  modified_base 20^21: mod_base = OTHER; note = Phosphorothioate Linkage
  modified_base 21: mod_base = OTHER; note = 2'-O-methyl nucleotide
  misc_feature 1..21: note = siRNA
tgatgttttgagcacctacta